European Patent Application EP 4 141 026 A1, published March 1, 2023. Title: Fusion proteins comprising anti C3b single domain antibody for complement regulation. Applicant: Aarhus University. The sequence listing filed with the application follows.

SEQUENCE LISTING (24 sequences)

SEQ ID NO: 1 - protein, 127 aa, Artificial Sequence
  Fusion protein
  MISC_FEATURE (1)..(127): EWE-hC3Nb1
MEWEQVQLVETGGGLVQAGGSLRLSCAASGSIFSINAMGWFRQAPGKEREFVATINRSGGRTYYADSVKGRFTISRDNGKNMVYLQMHSLKPEDTAIYYCAAGTGWSPQTDNEYNYWGQGTQVTVSS

SEQ ID NO: 2 - protein, 11 aa, Artificial Sequence
  CDR
  MISC_FEATURE (1)..(11): CDR1
SGSIFSINAMG

SEQ ID NO: 3 - protein, 10 aa, Artificial Sequence
  CDR
  MISC_FEATURE (1)..(10): CDR2
TINRSGGRTY

SEQ ID NO: 4 - protein, 14 aa, Artificial Sequence
  CDR
  MISC_FEATURE (1)..(14): CDR3
GTGWSPQTDNEYNY

SEQ ID NO: 5 - protein, 473 aa, Artificial Sequence
  Fusion protein
  MISC_FEATURE (1)..(473): EWEµH
EWEQVQLVETGGGLVQAGGSLRLSCAASGSIFSINAMGWFRQAPGKEREFVATINRSGGRTYYADSVKGRFTISRDNGKNMVYLQMHSLKPEDTAIYYCAAGTGWSPQTDNEYNYWGQGTQVTVSSGGGGSGGGGSGGGGSGGGGSRPCGHPGDTPFGTFTLTGGNVFEYGVKAVYTCNEGYQLLGEINYRECDTDGWTNDIPICEVVKCLPVTAPENGKIVSSAMEPDREYHFGQAVRFVCNSGYKIEGDEEMHCSDDGFWSKEKPKCVEISCKSPDVINGSPISQKIIYKENERFQYKCNMGYEYSERGDAVCTESGWRPLPSCEEAGGGGGGGGGGGGGKCGPPPPIDNGDITSFPLSVYAPASSVEYQCQNLYQLEGNKRITCRNGQWSEPPKCLHPCVISREIMENYNIALRWTAKQKLYSRTGESVEFVCKRGYRLSSRSHTLRTTCWDGKLEYPTCAKRENLYFQG

SEQ ID NO: 6 - protein, 20 aa, Artificial Sequence
  Linker
  MISC_FEATURE (1)..(20): Polypeptide linker connecting EWE-hC3Nb1 and the CCP2 domain of the factor H moiety
GGGGSGGGGSGGGGSGGGGS

SEQ ID NO: 7 - protein, 329 aa, Artificial Sequence
  Fusion protein
  MISC_FEATURE (1)..(329): EWEnH
EWEQVQLVETGGGLVQAGGSLRLSCAASGSIFSINAMGWFRQAPGKEREFVATINRSGGRTYYADSVKGRFTISRDNGKNMVYLQMHSLKPEDTAIYYCAAGTGWSPQTDNEYNYWGQGTQVTVSSGGGGSGGGGSGGGGSGGGGSRPCGHPGDTPFGTFTLTGGNVFEYGVKAVYTCNEGYQLLGEINYRECDTDGWTNDIPICEVVKCLPVTAPENGKIVSSAMEPDREYHFGQAVRFVCNSGYKIEGDEEMHCSDDGFWSKEKPKCVEISCKSPDVINGSPISQKIIYKENERFQYKCNMGYEYSERGDAVCTESGWRPLPSCEEA

SEQ ID NO: 8 - protein, 383 aa, Artificial Sequence
  Fusion protein
  MISC_FEATURE (1)..(383): Mini-FH
EDCNELPPRRNTEILTGSWSDQTYPEGTQAIYKCRPGYRSLGNIIMVCRKGEWVALNPLRKCQKRPCGHPGDTPFGTFTLTGGNVFEYGVKAVYTCNEGYQLLGEINYRECDTDGWTNDIPICEVVKCLPVTAPENGKIVSSAMEPDREYHFGQAVRFVCNSGYKIEGDEEMHCSDDGFWSKEKPKCVEISCKSPDVINGSPISQKIIYKENERFQYKCNMGYEYSERGDAVCTESGWRPLPSCEEAGGGGGGGGGGGGGKCGPPPPIDNGDITSFPLSVYAPASSVEYQCQNLYQLEGNKRITCRNGQWSEPPKCLHPCVISREIMENYNIALRWTAKQKLYSRTGESVEFVCKRGYRLSSRSHTLRTTCWDGKLEYPTCAK

SEQ ID NO: 9 - protein, 319 aa, Artificial Sequence
  Fusion protein
  MISC_FEATURE (1)..(319): µH comprising CCP2-CCP4 and CCP19-CCP20
RPCGHPGDTPFGTFTLTGGNVFEYGVKAVYTCNEGYQLLGEINYRECDTDGWTNDIPICEVVKCLPVTAPENGKIVSSAMEPDREYHFGQAVRFVCNSGYKIEGDEEMHCSDDGFWSKEKPKCVEISCKSPDVINGSPISQKIIYKENERFQYKCNMGYEYSERGDAVCTESGWRPLPSCEEAGGGGGGGGGGGGGKCGPPPPIDNGDITSFPLSVYAPASSVEYQCQNLYQLEGNKRITCRNGQWSEPPKCLHPCVISREIMENYNIALRWTAKQKLYSRTGESVEFVCKRGYRLSSRSHTLRTTCWDGKLEYPTCAK

SEQ ID NO: 10 - protein, 183 aa, Artificial Sequence
  Fusion protein
  MISC_FEATURE (1)..(183): nH comprising CCP2-CCP4
RPCGHPGDTPFGTFTLTGGNVFEYGVKAVYTCNEGYQLLGEINYRECDTDGWTNDIPICEVVKCLPVTAPENGKIVSSAMEPDREYHFGQAVRFVCNSGYKIEGDEEMHCSDDGFWSKEKPKCVEISCKSPDVINGSPISQKIIYKENERFQYKCNMGYEYSERGDAVCTESGWRPLPSCEEA

SEQ ID NO: 11 - protein, 61 aa, Homo sapiens
RPCGHPGDTPFGTFTLTGGNVFEYGVKAVYTCNEGYQLLGEINYRECDTDGWTNDIPICEV

SEQ ID NO: 12 - protein, 64 aa, Homo sapiens
VKCLPVTAPENGKIVSSAMEPDREYHFGQAVRFVCNSGYKIEGDEEMHCSDDGFWSKEKPKCVE

SEQ ID NO: 13 - protein, 57 aa, Homo sapiens
ISCKSPDVINGSPISQKIIYKENERFQYKCNMGYEYSERGDAVCTESGWRPLPSCEE

SEQ ID NO: 14 - protein, 59 aa, Homo sapiens
GKCGPPPPIDNGDITSFPLSVYAPASSVEYQCQNLYQLEGNKRITCRNGQWSEPPKCLH

SEQ ID NO: 15 - protein, 4 aa, Homo sapiens
PCVI

SEQ ID NO: 16 - protein, 61 aa, Homo sapiens
SREIMENYNIALRWTAKQKLYSRTGESVEFVCKRGYRLSSRSHTLRTTCWDGKLEYPTCAK

SEQ ID NO: 17 - protein, 13 aa, Artificial Sequence
  Linker
  MISC_FEATURE (1)..(13): Linker connecting CCP4-CCP19
AGGGGGGGGGGGG

SEQ ID NO: 18 - protein, 123 aa, Homo sapiens
KCGPPPPIDNGDITSFPLSVYAPASSVEYQCQNLYQLEGNKRITCRNGQWSEPPKCLHPCVISREIMENYNIALRWTAKQKLYSRTGESVEFVCKRGYRLSSRSHTLRTTCWDGKLEYPTCAK

SEQ ID NO: 19 - protein, 915 aa, Artificial Sequence
  Fusion protein
  MISC_FEATURE (1)..(915): C3b alpha chain sequence from rcsb.com [pdb id: 5O35] 749-1662
SNLDEDIIAEENIVSRSEFPESWLWNVEDLKEPPKNGISTKLMNIFLKDSITTWEILAVSMSDKKGICVADPFEVTVMQDFFIDLRLPYSVVRNEQVEIRAVLYNYRQNQELKVRVELLHNPAFCSLATTKRRHQQTVTIPPKSSLSVPYVIVPLKTGLQEVEVKAAVYHHFISDGVRKSLKVVPEGIRMNKTVAVRTLDPERLGREGVQKEDIPPADLSDQVPDTESETRILLQGTPVAQMTEDAVDAERLKHLIVTPSGCGEQNMIGMTPTVIAVHYLDETEQWEKFGLEKRQGALELIKKGYTQQLAFRQPSSAFAAFVKRAPSTWLTAYVVKVFSLAVNLIAIDSQVLCGAVKWLILEKQKPDGVFQEDAPVIHQEMIGGLRNNNEKDMALTAFVLISLQEAKDICEEQVNSLPGSITKAGDFLEANYMNLQRSYTVAIAGYALAQMGRLKGPLLNKFLTTAKDKNRWEDPGKQLYNVEATSYALLALLQLKDFDFVPPVVRWLNEQRYYGGGYGSTQATFMVFQALAQYQKDAPDHQELNLDVSLQLPSRSSKITHRIHWESASLLRSEETKENEGFTVTAEGKGQGTLSVVTMYHAKAKDQLTCNKFDLKVTIKPAPETEKRPQDAKNTMILEICTRYRGDQDATMSILDISMMTGFAPDTDDLKQLANGVDRYISKYELDKAFSDRNTLIIYLDKVSHSEDDCLAFKVHQYFNVELIQPGAVKVYAYYNLEESCTRFYHPEKEDGKLNKLCRDELCRCAEENCFIQKSDDKVTLEERLDKACEPGVDYVYKTRLVKVQLSNDFDEYIMAIEQTIKSGSDEVQVGQQRTFISPIKCREALKLEEKKHYLMWGLSSDFWGEKPNLSYIIGKDTWVEHWPEEDECQDEENQKQCQDLGAFTESMVVFGCPN

SEQ ID NO: 20 - protein, 105 aa, Homo sapiens
FFIDLRLPYSVVRNEQVEIRAVLYNYRQNQELKVRVELLHNPAFCSLATTKRRHQQTVTIPPKSSLSVPYVIVPLKTGLQEVEVKAAVYHHFISDGVRKSLKVVP

SEQ ID NO: 21 - protein, 64 aa, Homo sapiens
EDCNELPPRRNTEILTGSWSDQTYPEGTQAIYKCRPGYRSLGNIIMVCRKGEWVALNPLRKCQK

SEQ ID NO: 22 - protein, 565 aa, Homo sapiens
KVTYTSQEDLVEKKCLAKKYTHLSCDKVFCQPWQRCIEGTCVCKLPYQCPKNGTAVCATNRRSFPTYCQQKSLECLHPGTKFLNNGTCTAEGKFSVSLKHGNTDSEGIVEVKLVDQDKTMFICKSSWSMREANVACLDLGFQQGADTQRRFKLSDLSINSTECLHVHCRGLETSLAECTFTKRRTMGYQDFADVVCYTQKADSPMDDFFQCVNGKYISQMKACDGINDCGDQSDELCCKACQGKGFHCKSGVCIPSQYQCNGEVDCITGEDEVGCAGFASVTQEETEILTADMDAERRRIKSLLPKLSCGVKNRMHIRRKRIVGGKRAQLGDLPWQVAIKDASGITCGGIYIGGCWILTAAHCLRASKTHRYQIWTTVVDWIHPDLKRIVIEYVDRIIFHENYNAGTYQNDIALIEMKKDGNKKDCELPRSIPACVPWSPYLFQPNDTCIVSGWGREKDNERVFSLQWGEVKLISNCSKFYGNRFYEKEMECAGTYDGSIDACKGDSGGPLVCMDANNVTYVWGVVSWGENCGKPEFPGVYTKVANYFDWISYHVGRPFISQYNV

SEQ ID NO: 23 - protein, 124 aa, Artificial Sequence
  hC3Nb1
  MISC_FEATURE (1)..(124): hC3Nb1
MQVQLVETGGGLVQAGGSLRLSCAASGSIFSINAMGWFRQAPGKEREFVATINRSGGRTYYADSVKGRFTISRDNGKNMVYLQMHSLKPEDTAIYYCAAGTGWSPQTDNEYNYWGQGTQVTVSS

SEQ ID NO: 24 - protein, 645 aa, Artificial Sequence
  C3b
  MISC_FEATURE (1)..(645): C3b sequence from rcsb.com [pdb id: 5O35] 23-667
SPMYSIITPNILRLESEETMVLEAHDAQGDVPVTVTVHDFPGKKLVLSSEKTVLTPATNHMGNVTFTIPANREFKSEKGRNKFVTVQATFGTQVVEKVVLVSLQSGYLFIQTDKTIYTPGSTVLYRIFTVNHKLLPVGRTVMVNIENPEGIPVKQDSLSSQNQLGVLPLSWDIPELVNMGQWKIRAYYENSPQQVFSTEFEVKEYVLPSFEVIVEPTEKFYYIYNEKGLEVTITARFLYGKKVEGTAFVIFGIQDGEQRISLPESLKRIPIEDGSGEVVLSRKVLLDGVQNPRAEDLVGKSLYVSATVILHSGSDMVQAERSGIPIVTSPYQIHFTKTPKYFKPGMPFDLMVFVTNPDGSPAYRVPVAVQGEDTVQSLTQGDGVAKLSINTHPSQKPLSITVRTKKQELSEAEQATRTMQALPYSTVGNSNNYLHLSVLRTELRPGETLNVNFLLRMDRAHEAKIRYYTYLIMNKGRLLKAGRQVREPGQDLVVLPLSITTDFIPSFRLVAYYTLIGASGQREVVADSVWVDVKDSCVGSLVVKSGQSEDRQPVPGQQMTLKIEGDHGARVVLVAVDKGVFVLNKKNKLTQSKIWDVVEKADIGCTPGSGKDYAGVFSDAGLTFTSSSGQQTAQRAELQCPQPAA